European Patent Application EP 4 353 268 A1, published April 17, 2024. Title: Nanoparticle Comprising Peptide-Lipid Conjugate for Delivering Oligonucleotide into Target Cell and Pharmaceutical Composition Comprising Thereof. Applicant: NIBEC Co., Ltd. Seoul National University R&DB Foundation. The sequence listing filed with the application follows.

SEQUENCE LISTING (24 sequences)

SEQ ID NO: 1 - protein, 16 aa, Artificial Sequence
  RNA binding peptide
LKKLLKLLKKLLKLAG

SEQ ID NO: 2 - protein, 17 aa, Artificial Sequence
  RNA binding peptide
IKKILIKIIKKLIKLAG

SEQ ID NO: 3 - protein, 16 aa, Artificial Sequence
  RNA binding peptide
LRRLLRLLRRLLRLAG

SEQ ID NO: 4 - protein, 14 aa, Artificial Sequence
  RNA binding peptide
LKKLLKLLKLLLAG

SEQ ID NO: 5 - protein, 14 aa, Artificial Sequence
  RNA binding peptide
LRRLLRLLRLLLAG

SEQ ID NO: 6 - protein, 14 aa, Artificial Sequence
  RNA binding peptide
LRKIIRLIKLLLAG

SEQ ID NO: 7 - protein, 15 aa, Artificial Sequence
  RNA binding peptide
LKKLLKLLKLLKLAG

SEQ ID NO: 8 - protein, 16 aa, Artificial Sequence
  RNA binding peptide
WKKLLKLLKKLLKLAG

SEQ ID NO: 9 - protein, 16 aa, Artificial Sequence
  RNA binding peptide
WRRLLRLLRRLLRLAG

SEQ ID NO: 10 - protein, 16 aa, Artificial Sequence
  RNA binding peptide
WRKLLRLLKKLLKLAG

SEQ ID NO: 11 - protein, 15 aa, Artificial Sequence
  RNA binding peptide
LKKLLLLKKLLKWAG

SEQ ID NO: 12 - protein, 15 aa, Artificial Sequence
  RNA binding peptide
LRRLLLLRRLLRWAG

SEQ ID NO: 13 - protein, 15 aa, Artificial Sequence
  RNA binding peptide
LKRLIIIKKLIKWAG

SEQ ID NO: 14 - protein, 14 aa, Artificial Sequence
  RNA binding peptide
LKKLLKWLKLLLAG

SEQ ID NO: 15 - protein, 14 aa, Artificial Sequence
  RNA binding peptide
LRRLLRWLRLLLAG

SEQ ID NO: 16 - protein, 7 aa, Artificial Sequence
  peptide thatt bind to target cell surface
CAIYPRH

SEQ ID NO: 17 - RNA, 1461 nt, Artificial Sequence
  KRAS mRNA
auggaaguccaauuguuggaaucugggggugggcuuguccaaccuggugguucacuccgucugagcugcgccgcuuccggauucacuuucuccaccuuuucuaugaauuggguucgccaggccccaggcaagggacuugaguggguuagcuauaucagcaggaccaguaaaaccaucuacuacgccgacagcguuaagggaagguucacuauaucccgggacaauucuaagaauacuuuguacuugcaaaugaacucuuugcgggcagaagauacugcugucuacuauugugcacgagguagguuuuuugauuauuggggucaggggacccucguaaccguuuccagugggggcagcgaggguaagagcuccgguucagggucagaaucuaaaagcacugguggcuccgauauacaaaugacccagaguccaagcucucuuucagccagcgugggagacagggugaccaucaccugucgagcaucucaauccauuucaucauaccucaauugguaucaacagaagccuggggaagcaccaaaguugcuuauuuauucugccagcguacugcaaaguggcguaccuucccgcuucuccgggucugggaguggcacugauuuuacccucacaauuagcagccugcaacccgaggacuucgcuacauacuacugccaacaaaguguaaugauacccaugacauucgggcaaggcacaaaagucgagauaaagggaaguggaggagguggcucuaugccccgccgcgcugagaacugggaugaggccgaaguuggugcugaagaggccggaguugaagaauaugggccagaagaagauggcggugaggaaagcggggcugaagagagcgguccagaggagucugguccagaggaacuuggagcugaggaggagauggaggccggacguccacguccuguccugcgaucaguuaacucaagggagcccucacagguuaucuuuuguaaucgaagcccucgcgugguuuugcccgucuggcucaacuucgauggugaaccccaaccauacccaacccuccccccugguaccgggcggaggauucauuccuaucggggacaccuuuggcucuuccgagacgcugggacucacgauggccuguuggucaaucagaccgaacuguuugugcccagccugaacguagacgggcagccaauuuucgcaaacauaacacugcccguauauacauugaaagaaaggugucuucaggugguacgcagucugguuaaaccagaaaacuauaggcgucuggauaucgugcgcagccucuaugaggaccuugaagaccacccuaacgugcaaaaggaccucgagcggcucacucaggagcgcauagcucaucagcgcaugggagaugaaaaccuuuacuuucagggugggagcggcggcagcggcgggagucaucaucaccaucaucaucaccacuga

SEQ ID NO: 18 - RNA, 1398 nt, Artificial Sequence
  KRAS mRNA
auggaagugcaacuucucgaaucuggagggggguugguacaacccggcggcagcuugcgcuuguccugugcugccaguggguucacauuuucuacauucucuaugaacuggguuagacaagccccuggcaaagggcuggaaugggugagcuauauaagucgcaccuccaaaacuauuuacuaugcagauagugucaagggacgauuuacuaucagcagagauaacucuaagaacacucuguaucuccagaugaauucccuucgagccgaagacaccgcaguauauuacugugcuagagggcgcuucuucgacuacugggggcaaggcacucugguaacugucaguagcggggguucugagggcaaaaguucaggaucuggguccgagucuaagucaacuggcgggagcgacauacaaaugacucagagccccaguagccugagcgccuccguuggugacagagucacuauuacaugucgggcaucucaaucuauuuccucuuaucuuaacugguaucagcaaaagccaggcgaagcccccaaacuccugauauacuccgcuaguguucuucagaguggcguuccuagucgcuucagcggauccggaaguggcacugauuuuacacuuacaauuaguuccuugcagccugaagauuuugccacauacuacugucagcaaucagucaugauucccaugaccuuugggcaagggaccaaaguugagaucaaaggcuccggaggaggagggucuauggaaaacagauggcaaguuaugaucguuuggcaaguagaucguaugcgaauacgcacauggaaaucacugguaaagcaccacauguaugugucaggcaaagcacgaggaugguuuuaucgucaucacuaugagucaccacauccccgcaucagcucugaggugcacauaccacucggugaugcucgucuggucauaacuaccuacuggggccuccacacuggugaaagagauuggcaccucggccaaggaguaaguauagaauggcgcaaaaagcguuauucaacccaaguggauccugaguuggcagaucaguugauccacuuguauuacuuugacugcuucagcgauagugcuauucggaaggcccuccucgggcacauuguaagcccacggugcgaguaucaagcuggucauaacaagguugguagccuccaguacuuggcuuuggcugcacuuauaacacccaaaaagauaaaaccuccacuccccucagugacuaaacucacugaggaucguuggaacaaaccccagaaaaccaaggggcacagggguucacacaccaugaauggccacgagaauuuguauuuccaagggggauccgggggcaguggagggucucaccaucaucaccaccaccaccauuga

SEQ ID NO: 19 - RNA, 19 nt, Artificial Sequence
  KRAS siRNA
cagcuaauucagaaucauu

SEQ ID NO: 20 - RNA, 19 nt, Artificial Sequence
  KRAS siRNA
aaugauucugaauuagcug

SEQ ID NO: 21 - DNA, 20 bp, Artificial Sequence
  primer
tgacctgctgtgtcgagaat

SEQ ID NO: 22 - DNA, 21 bp, Artificial Sequence
  primer
ttgtggacgaatatgatccaa

SEQ ID NO: 23 - DNA, 20 bp, Artificial Sequence
  primer
cgccgctagaggtgaaattc

SEQ ID NO: 24 - DNA, 19 bp, Artificial Sequence
  primer
ttggcaaatgctttcgctc